European Patent Specification EP 3 470 421 B9, published October 4, 2023. Title: CHIMERIC IL-1 RECEPTOR TYPE I AGONISTS AND ANTAGONISTS. Applicant: ELEVEN BIOTHERAPEUTICS, INC. Application EP11749612.5. The sequence listing filed with the application follows.

SEQUENCE LISTING (58 sequences)

SEQ ID NO: 1 - protein, 153 aa, Homo sapiens
APVRSLNCTLRDSQQKSLVMSGPYELKALHLQGQDMEQQVVFSMSFVQGEESNDKIPVALGLKEKNLYLSCVLKDDKPTLQLESVDPKNYPKKKMEKRFVFNKIEINNKLEFESAQFPNWYISTSQAENMPVFLGGTKGGQDITDFTMQFVSS

SEQ ID NO: 2 - protein, 159 aa, Homo sapiens
SAPFSFLSNVKYNFMRIIKYEFILNDALNQSIIRANDQYLTAAALHNLDEAVKFDMGAYKSSKDDAKITVILRISKTQLYVTAQDEDQPVLLKEMPEIPKTITGSETNLLFFWETHGTKNYFTSVAHPNLFIATKQDYWVCLAGGPPSITDFQILENQA

SEQ ID NO: 3 - protein, 151 aa, Homo sapiens
RPSGRKSSKMQAFRIWDVNQKTFYLRNNQLVAGYLQGPNVNLEEKIDVVPIEPHALFLGIHGGKMCLSCVKSGDETRLQLEAVNITDLSENRKQDKRFAFIRSDSGPTTSFESAACPGWFLCTAMEADQPVSLTNMPDEGVMVTKFYFQED

SEQ ID NO: 4 - protein, 160 aa, Homo sapiens
SSITGISPITEYLASLSTYNDQSITFALEDESYEIYVEDLKKDEKKDKVLLSYYESQHPSNESGDGVDGKMLMVTLSPTKDFWLHANNKEHSVELHKCEKPLPDQAFFVLHNMHSNCVSFECKTDPGVFIGVKDNHLALIKVDSSENLCTENILFKLSET

SEQ ID NO: 5 - protein, 154 aa, Homo sapiens
VLSGALCFRMKDSALKVLYLHNNQLLAGGLHAGKVIKGEEISVVPNRWLDASLSPVILGVQGGSQCLSCGVGQEPTLTLEPVNIMELYLGAKESKSFTFYRRDMGLTSSFESAAYPGWFLCTVPEADQPVRLTQLPENGGWNAPITDFYFQQCD

SEQ ID NO: 6 - protein, 158 aa, Homo sapiens
MEKALKIDTPQQGSIQDINHRVWVLQDQTLIAVPRKDRMSPVTIALISCRHVETLEKDRGNPIYLGLNGLNLCLMCAKVGDQPTLQLKEKDIMDLYNQPEPVKSFLFYHSQSGRNSTFESVAFPGWFIAVSSEGGCPLILTQELGKANTTDFGLTMLF

SEQ ID NO: 7 - protein, 157 aa, Homo sapiens
MNPQREAAPKSYAIRDSRQMVWVLSGNSLIAAPLSRSIKPVTLHLIACRDTEFSDKEKGNMVYLGIKGKDLCLFCAEIQGKPTLQLKEKNIMDLYVEKKAQKPFLFFHNKEGSTSVFQSVSYPGWFIATSTTSGQPIFLTKERGITNNTNFYLDSVE

SEQ ID NO: 8 - protein, 169 aa, Homo sapiens
MRGTPGDADGGGRAVYQSMCKPITGTINDLNQQVWTLQGQNLVAVPRSDSVTPVTVAVITCKYPEALEQGRGDPIYLGIQNPEMCLYCEKVGEQPTLQLKEQKIMDLYGQPEPVKPFLFYRAKTGRTSTLESVAFPDWFIASSKRDQPIILTSELGKSYNTAFELNIND

SEQ ID NO: 9 - protein, 25 aa, Homo sapiens
WDVNQKTFYLRNNQLVAGYLQGPNV

SEQ ID NO: 10 - protein, 5 aa, Homo sapiens
NLEEK

SEQ ID NO: 11 - protein, 32 aa, Homo sapiens
RIWDVNQKTFYLRNNQLVAGYLQGPNVNLEEK

SEQ ID NO: 12 - protein, 7 aa, Homo sapiens
AMEADQP

SEQ ID NO: 13 - protein, 28 aa, Homo sapiens
FLCTAMEADQPVSLTNMPDEGVMVTKFY

SEQ ID NO: 14 - protein, 10 aa, Homo sapiens
VQGEESNDKI

SEQ ID NO: 15 - protein, 8 aa, Homo sapiens
KKKMEKRF

SEQ ID NO: 16 - protein, 73 aa, Homo sapiens
FSMSFVQGEESNDKIPVALGLKEKNLYLSCVLKDDKPTLQLESVDPKNYPKKKMEKRFVFNKIEINNKLEFES

SEQ ID NO: 17 - protein, 153 aa, Artificial Sequence
  Synthetic polypeptide
APVRSLAFRIWDVNQKTFYLRNNQLVAGYLQGPNVNLEEKIDVSFVQGEESNDKIPVALGIHGGKMCLSCVKSGDETRLQLEAVDPKNYPKKKMDKRFAFIRSDSGPTTSFESAACPGWFLCTAMEADQPVSLTNMPDEGVMVTKFYMQFVSS

SEQ ID NO: 18 - protein, 153 aa, Artificial Sequence
  Synthetic polypeptide
APVRSLAFRIWDVNQKTFYLRNNQLVAGYLQGPNVNLEEKIDVSFVQGEESNDKIPVALGIHGGKMCLSCVKSGDETRLQLEAVDPKNYPKKKMEKRFVFNKIEINNKLSFESAACPGWFLCTAMEADQPVSLTNMPDEGVMVTKFYMQFVSS

SEQ ID NO: 19 - protein, 153 aa, Artificial Sequence
  Synthetic polypeptide
APVRSLAFRIWDVNQKTFYLRNNQLVAGYLQGPNVNLEEKFSMSFVQGEESNDKIPVALGLKEKNLYLSCVLKDDKPTLQLESVDPKNYPKKKMEKRFVFIRSDSGPTTSFESAACPGWFLCTAMEADQPVSLTNMPDEGVMVTKFTMQFVSS

SEQ ID NO: 20 - protein, 153 aa, Artificial Sequence
  Synthetic polypeptide
APVRSLAFRIWDVNQKTFYLRNNQLVAGYLQGPNVNLEEKFSMSFVQGEESNDKIPVALGLKEKNLYLSCVLKDDKPTLQLESVDPKNYPKKKMEKRFVFNKIEINNKLEFESAACPGWFLCTAMEADQPVSLTNMPDEGVMVTKFTMQFVSS

SEQ ID NO: 21 - protein, 153 aa, Artificial Sequence
  Synthetic polypeptide
APVRSLNCRIWDVNQKTFYLRNNQLVAGYLQGPNVNLEEKFSMSFVQGEESNDKIPVALGLKEKNLYLSCVLKDDKPTLQLESVDPKNYPKKKMEKRFVFNKIEINNKLEFESAQFPNWFLCTAMEADQPVSLTNMPDEGVMVTKFYMQFVSS

SEQ ID NO: 22 - protein, 11 aa, Artificial Sequence
  Synthetic peptide
DICLPRWGCLW

SEQ ID NO: 23 - protein, 152 aa, Artificial Sequence
  Synthetic peptide
APVRSLNCTLWDVNQKTFYLRNNQLVAGYLQGPNVEQQVVFSMSFVQGEESNDKIPVALGLKEKNLYLSCVLKDDKPTLQLESVDPKNYPKKKMEKRFVFNKIEINNKLEFESAQFPNWYISTSMEADQPVFLGGTKGGQDITDFTMQFVSS

SEQ ID NO: 24 - protein, 153 aa, Artificial Sequence
  Synthetic polypeptide
APVRSLNCRIWDVNQKTFYLRNNQLVAGYLQGPNVNLEEKFSMSFVQGEESNDKIPVALGLKEKNLYLSCVLKDDKPTLQLESVDPKNYPKKKMEKRFVFNKIEINNKLEFESAQFPNWFLCTAMEADQPVSLTNMPDEGQDITDFTMQFVSS

SEQ ID NO: 25 - DNA, 459 bp, Artificial Sequence
  Synthetic polynucleotide
gcacctgtacgatcactggccttcagaatctgggatgttaaccagaagaccttctatctgaggaacaaccaactagttgctggatacttgcaaggaccaaatgtcaatttagaagaaaagatagatgtgtcctttgtacaaggagaagaaagtaatgacaaaatacctgtggccttgggcatccatggagggaagatgtgcctgtcctgtgtcaagtctggtgatgagaccagactccagctggaggcagttgatcccaaaaattacccaaagaagaagatggacaagcgcttcgccttcatccgctcagacagcggccccaccaccagttttgagtctgccgcctgccccggttggttcctctgcacagcgatggaagctgaccagcccgtcagcctcaccaatatgcctgacgaaggcgtcatggtcaccaaattctacatgcaatttgtgtcttcc

SEQ ID NO: 26 - DNA, 459 bp, Artificial Sequence
  Synthetic polynucleotide
gcacctgtacgatcactggccttcagaatctgggatgttaaccagaagaccttctatctgaggaacaaccaactagttgctggatacttgcaaggaccaaatgtcaatttagaagaaaagatagatgtgtcctttgtacaaggagaagaaagtaatgacaaaatacctgtggccttgggcatccatggagggaagatgtgcctgtcctgtgtcaagtctggtgatgagaccagactccagctggaggcagttgatcccaaaaattacccaaagaagaagatggaaaagcgatttgtcttcaacaagatagaaatcaataacaagctgagttttgagtctgccgcctgccccggttggttcctctgcacagcgatggaagctgaccagcccgtcagcctcaccaatatgcctgacgaaggcgtcatggtcaccaaattctacatgcaatttgtgtcttcc

SEQ ID NO: 27 - DNA, 459 bp, Artificial Sequence
  Synthetic polynucleotide
gcacctgtacgatcactggccttcagaatctgggatgttaaccagaagaccttctatctgaggaacaaccaactagttgctggatacttgcaaggaccaaatgtcaatttagaagaaaagttctccatgtcctttgtacaaggagaagaaagtaatgacaaaatacctgtggccttgggcctcaaggaaaagaatctgtacctgtcctgcgtgttgaaagatgataagcccactctacagctggagagtgtagatcccaaaaattacccaaagaagaagatggaaaagcgatttgtcttcatccgctcagacagcggccccaccaccagttttgagtctgccgcctgccccggttggttcctctgcacagcgatggaagctgaccagcccgtcagcctcaccaatatgcctgacgaaggcgtcatggtcaccaaattcaccatgcaatttgtgtcttcc

SEQ ID NO: 28 - DNA, 459 bp, Artificial Sequence
  Synthetic polynucleotide
gcacctgtacgatcactggccttcagaatctgggatgttaaccagaagaccttctatctgaggaacaaccaactagttgctggatacttgcaaggaccaaatgtcaatttagaagaaaagttctccatgtcctttgtacaaggagaagaaagtaatgacaaaatacctgtggccttgggcctcaaggaaaagaatctgtacctgtcctgcgtgttgaaagatgataagcccactctacagctggagagtgtagatcccaaaaattacccaaagaagaagatggaaaagcgatttgtcttcaacaagatagaaatcaataacaagctggaatttgagtctgccgcctgccccggttggttcctctgcacagcgatggaagctgaccagcccgtcagcctcaccaatatgcctgacgaaggcgtcatggtcaccaaattcaccatgcaatttgtgtcttcc

SEQ ID NO: 29 - DNA, 459 bp, Artificial Sequence
  Synthetic polynucleotide
gcacctgtacgatcactgaactgcagaatctgggatgttaaccagaagaccttctatctgaggaacaaccaactagttgctggatacttgcaaggaccaaatgtcaatttagaagaaaagttctccatgtcctttgtacaaggagaagaaagtaatgacaaaatacctgtggccttgggcctcaaggaaaagaatctgtacctgtcctgcgtgttgaaagatgataagcccactctacagctggagagtgtagatcccaaaaattacccaaagaagaagatggaaaagcgatttgtcttcaacaagatagaaatcaataacaagctggaatttgagtctgcccagttccccaactggttcctctgcacagcgatggaagctgaccagcccgtcagcctcaccaatatgcctgacgaaggcgtcatggtcaccaaattctacatgcaatttgtgtcttcc

SEQ ID NO: 30 - DNA, 456 bp, Artificial Sequence
  Synthetic polynucleotide
gcacctgtacgatcactgaactgcacgctctgggatgttaaccagaagaccttctatctgaggaacaaccaactagttgctggatacttgcaaggaccaaatgtcgagcaacaagtggtgttctccatgtcctttgtacaaggagaagaaagtaatgacaaaatacctgtggccttgggcctcaaggaaaagaatctgtacctgtcctgcgtgttgaaagatgataagcccactctacagctggagagtgtagatcccaaaaattacccaaagaagaagatggaaaagcgatttgtcttcaacaagatagaaatcaataacaagctggaatttgagtctgcccagttccccaactggtacatcagcacctctatggaagctgaccagcccgtcttcctgggagggaccaaaggcggccaggatataactgacttcaccatgcaatttgtgtcttcc

SEQ ID NO: 31 - DNA, 459 bp, Artificial Sequence
  Synthetic polynucleotide
gcacctgtacgatcactgaactgcagaatctgggatgttaaccagaagaccttctatctgaggaacaaccaactagttgctggatacttgcaaggaccaaatgtcaatttagaagaaaagttctccatgtcctttgtacaaggagaagaaagtaatgacaaaatacctgtggccttgggcctcaaggaaaagaatctgtacctgtcctgcgtgttgaaagatgataagcccactctacagctggagagtgtagatcccaaaaattacccaaagaagaagatggaaaagcgatttgtcttcaacaagatagaaatcaataacaagctggaatttgagtctgcccagttccccaactggttcctctgcacagcgatggaagctgaccagcccgtcagcctcaccaatatgcctgacgaaggccaggatataactgacttcaccatgcaatttgtgtcttcc

SEQ ID NO: 32 - protein, 153 aa, Artificial Sequence
  Synthetic polypeptide
APVRSLAFRIWDVNQKTFYLRNNQLVAGYLQGPNVNLEEKFSMSFVQGEESNDKIPVALGLKEKNLYLSCVLKDDKPTLQLESVDPKNYPKKKMEKRFVFNKIEINNKLEFESAQFPNWFLCTAMEADQPVSLTNMPDEGVMVTKFYMQFVSS

SEQ ID NO: 33 - protein, 153 aa, Artificial Sequence
  Synthetic polypeptide
APVRSQAFRIWDVNQKTFYLRNNQLVAGYLQGPNVNLEEKFSMSFVQGEESNDKIPVALGLKEKNLYLSCVLKDDKPTLQLESVDPKNYPKKKMEKRFVFNKIEINNKLEFESAQFPNWFLCTAMEADQPVSLTNMPDEGVMVTKFYMQFVSS

SEQ ID NO: 34 - protein, 153 aa, Artificial Sequence
  Synthetic polypeptide
APVRSLAFRIWDVNQKTFYLRNNQLVAGYLQGPNVNLEEKIDVSFVQGEESNDKIPVALGLKEKNLYLSCVLKDDKPTLQLESVDPKNYPKKKMEKRFVFNKIEINNKLEFESAQFPNWFLCTAMEADQPVSLTNMPDEGVMVTKFYMQFVSS

SEQ ID NO: 35 - protein, 153 aa, Artificial Sequence
  Synthetic polypeptide
APVRSLNCRIWDVNQKTFYLRNNQLVAGYLQGPNVNLEEKIDVSFVQGEESNDKIPVALGLKEKNLYLSCVLKDDKPTLQLESVDPKNYPKKKMEKRFVFNKIEINNKLEFESAQFPNWFLCTAMEADQPVSLTNMPDEGVMVTKFYMQFVSS

SEQ ID NO: 36 - protein, 153 aa, Artificial Sequence
  Synthetic polypeptide
APVRSLNCRIWDVNQKTFYLRNNQLVAGYLQGPNVNLEEKFSMSFVQGEESNDKIPVALGLKEKNLYLSCVLKDDKPTLQLESVDPKNYPKKKMEKRFVFNKIEINNKLEFESAQFPNWFLCTAMEADQPVSLTNMPDEGVMVTKFTMQFVSS

SEQ ID NO: 37 - protein, 151 aa, Artificial Sequence
  Synthetic polypeptide
APVRSLAFRIWDVNQKTFYLRNNQLVAGYLQGPNVNLEEKFSMSFVQGEESNDKIPVALGLKEKNLYLSCVLKDDKPTLQLESVDPKNYPKKKMEKRFVFNKIEINNKLEFESAQFPNWFLCTAMEADQPVSLTNMPDEGVMVTKFYFQED

SEQ ID NO: 38 - protein, 151 aa, Artificial Sequence
  Synthetic polypeptide
APVRSLNCRIWDVNQKTFYLRNNQLVAGYLQGPNVNLEEKFSMSFVQGEESNDKIPVALGLKEKNLYLSCVLKDDKPTLQLESVDPKNYPKKKMEKRFVFNKIEINNKLEFESAQFPNWFLCTAMEADQPVSLTNMPDEGVMVTKFYFQED

SEQ ID NO: 39 - protein, 165 aa, Artificial Sequence
  Synthetic polypeptide
SAPFSFLSNVKYNFMRIIKYEFRIWDVNQKTFYLRNNQLVAGYLQGPNVNLEEKFDMGAYKSSKDDAKITVILRISKTQLYVTAQDEDQPVLLKEMPEIPKTITGSETNLLFFWETHGTKNYFTSVAHPNLFLCTAMEADQPVSLTNMPDEGVMVTKFYILENQA

SEQ ID NO: 40 - protein, 160 aa, Artificial Sequence
  Synthetic polypeptide
DKPTLQLESVDPKNYPKKKMEKRFVFNKIEINNKLEFESAQFPNWFLCTAMEADQPVSLTNMPDEGVMVTKFYMQFVSSGGSGGGSAPVRSLNCRIWDVNQKTFYLRNNQLVAGYLQGPNVNLEEKFSMSFVQGEESNDKIPVALGLKEKNLYLSCVLKD

SEQ ID NO: 41 - protein, 160 aa, Artificial Sequence [sequence omitted]

SEQ ID NO: 42 - protein, 6 aa, Artificial Sequence
  Synthetic 6xHis tag
HHHHHH

SEQ ID NO: 43 - protein, 7 aa, Homo sapiens
YLQGPNV

SEQ ID NO: 44 - protein, 8 aa, Homo sapiens
MEADQPVS

SEQ ID NO: 45 - protein, 6 aa, Homo sapiens
RSLAFR

SEQ ID NO: 46 - protein, 6 aa, Homo sapiens
IDVSFV

SEQ ID NO: 47 - protein, 6 aa, Homo sapiens
KKMDKR

SEQ ID NO: 48 - protein, 6 aa, Homo sapiens
KFYMQF

SEQ ID NO: 49 - protein, 6 aa, Homo sapiens
NKLSFE

SEQ ID NO: 50 - protein, 6 aa, Homo sapiens
EEKFSM

SEQ ID NO: 51 - protein, 6 aa, Homo sapiens
RFVFIR

SEQ ID NO: 52 - protein, 6 aa, Homo sapiens
VTKFTM

SEQ ID NO: 53 - protein, 6 aa, Homo sapiens
FESAAC

SEQ ID NO: 54 - protein, 6 aa, Homo sapiens
VTKFTM

SEQ ID NO: 55 - protein, 6 aa, Homo sapiens
LNCRIW

SEQ ID NO: 56 - protein, 6 aa, Homo sapiens
PNWFLC

SEQ ID NO: 57 - protein, 141 aa, Artificial Sequence
  Synthetic polypeptide consensus sequence
  Variant (2)..(3): Xaa can be any amino acid
  Variant (6)..(13): Xaa can be any amino acid
  misc_feature (14)..(14): Xaa can be any amino acid or absent
  Variant (17)..(18): Xaa can be any amino acid
  Variant (22)..(39): Xaa can be any amino acid
  misc_feature (40)..(49): Xaa can be any amino acid or absent
  Variant (52)..(58): Xaa can be any amino acid
  Variant (63)..(65): Xaa can be any amino acid
  Variant (67)..(69): Xaa can be any amino acid
  Variant (74)..(74): Xaa can be any amino acid
  Variant (76)..(83): Xaa can be any amino acid
  misc_feature (84)..(84): Xaa can be any amino acid or absent
  Variant (86)..(87): Xaa can be any amino acid
  Variant (91)..(91): Xaa can be any amino acid
  Variant (93)..(102): Xaa can be any amino acid
  Variant (107)..(108): Xaa can be any amino acid
  Variant (110)..(110): Xaa can be any amino acid
  Variant (112)..(114): Xaa can be any amino acid
  Variant (116)..(121): Xaa can be any amino acid
  Variant (124)..(124): Xaa can be any amino acid
  Variant (126)..(130): Xaa can be any amino acid
  misc_feature (131)..(131): Xaa can be any amino acid or absent
  Variant (133)..(135): Xaa can be any amino acid
  Variant (137)..(137): Xaa can be any amino acid
  Variant (139)..(140): Xaa can be any amino acid
DXXQKXXXXXXXXXLAXXLQGXXXXXXXXXXXXXXXXXXXXXXXXXXXXLGXXXXXXXLSCVXXXDXXXLQLEXVXXXXXXXXXKXXKRFXFXXXXXXXXXXFESAXXPXWXXXTXXXXXXPVXLXXXXXXGXXXTXFXXQ

SEQ ID NO: 58 - protein, 5 aa, Homo sapiens
APVRS